European Patent Application EP 4 285 924 A2, published December 6, 2023. Title: TREATING NON-ALCOHOLIC STEATOHEPATITIS (NASH) AND HEPATOCELLULAR CARCINOMA (HCC) WITH COMPOUNDS BINDING THE ECTODOMAIN OF PLATELET GLYCOPROTEIN IB (GPIB) ALPHA. Applicant: Deutsches Krebsforschungszentrum Stiftung des öffentlichen Rechts. The sequence listing filed with the application follows.

SEQUENCE LISTING (1 sequence)

SEQ ID NO: 1 - protein, 654 aa, homo sapiens
MPLLLLLLLLPSPLHPHPICEVSKVASHLEVNCDKRNLTALPPDLPKDTTILHLSENLLYTFSLATLMPYTRLTQLNLDRCELTKLQVDGTLPVLGTLDLSHNQLQSLPLLGQTLPALTVLDVSFNRLTSLPLGALRGLGELQELYLKGNELKTLPPGLLTPTPKLEKLSLANNNLTELPAGLLNGLENLDTLLLQENSLYTIPKGFFGSHLLPFAFLHGNPWLCNCEILYFRRWLQDNAENVYVWKQGVDVKAMTSNVASVQCDNSDKFPVYKYPGKGCPTLGDEGDTDLYDYYPEEDTEGDKVRATRTVVKFPTKAHTTPWGLFYSWSTASLDSQMPSSLHPTQESTKEQTTFPPRWTPNFTLHMESITFSKTPKSTTEPTPSPTTSEPVPEPAPNMTTLEPTPSPTTPEPTSEPAPSPTTPEPTSEPAPSPTTPEPTSEPAPSPTTPEPTPIPTIATSPTILVSATSLITPKSTFLTTTKPVSLLESTKKTIPELDQPPKLRGVLQGHLESSRNDPFLHPDFCCLLPLGFYVLGLFWLLFASVVLILLLSWVGHVKPQALDSGQGAALTTATQTTHLELQRGRQVTVPRAWLLFLRGSLPTFRSSLFLWVRPNGRVGPLVAGRRPSALSQGRGQDLLSTVSIRYSGHSLSL